European Patent Application EP 4 458 989 A1, published November 6, 2024. Title: KIT FOR IDENTIFYING TUMOR TISSUE-OF-ORIGIN AND DATA ANALYSIS METHOD. Applicant: Hangzhou ShengTing Medical Technology Ltd. The sequence listing filed with the application follows.

SEQUENCE LISTING (16 sequences)

SEQ ID NO: 1 - DNA, 27 bp, synthetic construct
  source 1..27: mol_type = other DNA; note = A01-T
  modified_base 1..25: mod_base = m5c
  modified_base 26: mod_base = s2c
ntnangangntntnngtntanaannnt

SEQ ID NO: 2 - DNA, 30 bp, synthetic construct
  source 1..30: mol_type = other DNA; note = A01-B
  modified_base 1..30: mod_base = m5c
ggttgtagatnggaagagnanangtntaan

SEQ ID NO: 3 - DNA, 28 bp, synthetic construct
  source 1..28: mol_type = other DNA; note = A02-T
  modified_base 1..26: mod_base = m5c
  modified_base 27: mod_base = s2c
ntanangngntntnngatntantnannt

SEQ ID NO: 4 - DNA, 31 bp, synthetic construct
  source 1..31: mol_type = other DNA; note = A02-B
  modified_base 11..31: mod_base = m5c
gtgagtagatnggaagagnanangtntgaan

SEQ ID NO: 5 - DNA, 28 bp, synthetic construct
  source 1..28: mol_type = other DNA; note = A03-T
  modified_base 1..19: mod_base = m5c
  modified_base 27: mod_base = s2c
ntanangngntntnngatntaggatgnt

SEQ ID NO: 6 - DNA, 31 bp, synthetic construct
  source 1..31: mol_type = other DNA; note = A03-B
  modified_base 1..31: mod_base = m5c
natnntagatnggaagagnanangtntgaan

SEQ ID NO: 7 - DNA, 29 bp, synthetic construct
  source 1..29: mol_type = other DNA; note = A04-T
  modified_base 1..27: mod_base = m5c
  modified_base 28: mod_base = s2c
ntananangntnttnngatntatngannt

SEQ ID NO: 8 - DNA, 31 bp, synthetic construct
  source 1..31: mol_type = other DNA; note = A04-B
  modified_base 1..31: mod_base = m5c
gtngatagatnggaagagnanangtntgaan

SEQ ID NO: 9 - DNA, 29 bp, synthetic construct
  source 1..29: mol_type = other DNA; note = A05-T
  modified_base 1..22: mod_base = m5c
  modified_base 28: mod_base = s2c
ntanangangntnttnngtntnaagagnt

SEQ ID NO: 10 - DNA, 31 bp, synthetic construct
  source 1..31: mol_type = other DNA; note = A05-B
  modified_base 1..31: mod_base = m5c
ntnttgagatnggaagagnanangtntgaan

SEQ ID NO: 11 - DNA, 29 bp, synthetic construct
  source 1..29: mol_type = other DNA; note = A06-T
  modified_base 1..27: mod_base = m5c
  modified_base 28: mod_base = s2c
ntanangangntnttnngatntnatannt

SEQ ID NO: 12 - DNA, 29 bp, synthetic construct
  source 1..29: mol_type = other DNA; note = A06-B
  modified_base 3..29: mod_base = m5c
gtnatgagatnggaagagnananntgaan

SEQ ID NO: 13 - DNA, 51 bp, synthetic construct
  source 1..51: PCR_primers = fwd_name:R01_F,fwd_seq:aatgatacggcgaccaccgcactctttccctacacgacgctcttccgatct,rev_name:R01_R,rev_seq:caagcagaagacggcatacgagattcgccttagtgagttcagacgtgtgctcttccgatct; mol_type = other DNA; note = upstream primer for R01
aatgatacggcgaccaccgcactctttccctacacgacgctcttccgatct

SEQ ID NO: 14 - DNA, 61 bp, synthetic construct
  source 1..61: PCR_primers = fwd_name:R01_F,fwd_seq:aatgatacggcgaccaccgcactctttccctacacgacgctcttccgatct,rev_name:R01_R,rev_seq:caagcagaagacggcatacgagattcgccttagtgagttcagacgtgtgctcttccgatct; mol_type = other DNA; note = downstream primer for R01
caagcagaagacggcatacgagattcgccttagtgagttcagacgtgtgctcttccgatct

SEQ ID NO: 15 - DNA, 54 bp, synthetic construct
  source 1..54: PCR_primers = fwd_name:R02_F,fwd_seq:aatgatacggcgaccaccgatacactctttccctacacgacgctcttccgatct,rev_name:R02_R,rev_seq:caagcagaagacggcatacgagatctagtacggtgtcagacgtgtgctcttccgatct; mol_type = other DNA; note = upstream primer for R02
aatgatacggcgaccaccgatacactctttccctacacgacgctcttccgatct

SEQ ID NO: 16 - DNA, 58 bp, synthetic construct
  source 1..58: PCR_primers = fwd_name:R02_F,fwd_seq:aatgatacggcgaccaccgatacactctttccctacacgacgctcttccgatct,rev_name:R02_R,rev_seq:caagcagaagacggcatacgagatctagtacggtgtcagacgtgtgctcttccgatct; mol_type = other DNA; note = downstream primer for R02
caagcagaagacggcatacgagatctagtacggtgtcagacgtgtgctcttccgatct